European Patent Specification EP 3 458 577 B1, published November 6, 2024. Title: NEW FATTY ACID DECARBOXYLASE AND ITS USES. Applicant: CEA CNRS. The sequence listing filed with the application follows.

SEQUENCE LISTING (32 sequences)

SEQ ID NO: 1 - protein, 594 aa, Chlorella variabilis
RASAVEDIRKVLSDSSSPVAGQKYDYILVGGGTAACVLANRLSADGSKRVLVLEAGPDNTSRDVKIPAAITRLFRSPLDWNLFSELQEQLAERQIYMARGRLLGGSSATNATLYHRGAAGDYDAWGVEGWSSEDVLSWFVQAETNADFGPGAYHGSGGPMRVENPRYTNKQLHTAFFKAAEEVGLTPNSDFNDWSHDHAGYGTFQVMQDKGTRADMYRQYLKPVLGRRNLQVLTGAAVTKVNIDQAAGKAQALGVEFSTDGPTGERLSAELAPGGEVIMCAGAVHTPFLLKHSGVGPSAELKEFGIPVVSNLAGVGQNLQDQPACLTAAPVKEKYDGIAISDHIYNEKGQIRKRAIASYLLGGRGGLTSTGCDRGAFVRTAGQALPDLQVRFVPGMALDPDGVSTYVRFAKFQSQGLKWPSGITMQLIACRPQSTGSVGLKSADPFAPPKLSPGYLTDKDGADLATLRKGIHWARDVARSSALSEYLDGELFPGSGVVSDDQIDEYIRRSIHSSNAITGTCKMGNAGDSSSVVDNQLRVHGVEGLRVVDASVVPKIPGGQTGAPVVMIAERAAALLTGKATIGASAAAPATVAA

SEQ ID NO: 2 - protein, 654 aa, Chlorella variabilis
MASITSRASARASCSQANTRAGRVALSGGALLRPARPARSFVPARKQQQGAVRRGGALSARASAVEDIRKVLSDSSSPVAGQKYDYILVGGGTAACVLANRLSADGSKRVLVLEAGPDNTSRDVKIPAAITRLFRSPLDWNLFSELQEQLAERQIYMARGRLLGGSSATNATLYHRGAAGDYDAWGVEGWSSEDVLSWFVQAETNADFGPGAYHGSGGPMRVENPRYTNKQLHTAFFKAAEEVGLTPNSDFNDWSHDHAGYGTFQVMQDKGTRADMYRQYLKPVLGRRNLQVLTGAAVTKVNIDQAAGKAQALGVEFSTDGPTGERLSAELAPGGEVIMCAGAVHTPFLLKHSGVGPSAELKEFGIPVVSNLAGVGQNLQDQPACLTAAPVKEKYDGIAISDHIYNEKGQIRKRAIASYLLGGRGGLTSTGCDRGAFVRTAGQALPDLQVRFVPGMALDPDGVSTYVRFAKFQSQGLKWPSGITMQLIACRPQSTGSVGLKSADPFAPPKLSPGYLTDKDGADLATLRKGIHWARDVARSSALSEYLDGELFPGSGVVSDDQIDEYIRRSIHSSNAITGTCKMGNAGDSSSVVDNQLRVHGVEGLRVVDASVVPKIPGGQTGAPVVMIAERAAALLTGKATIGASAAAPATVAA

SEQ ID NO: 3 - protein, 729 aa, artificial sequence
  shGMC
MGHHHHHHSDKIIHLTDDSFDTDVLKADGAILVDFWAEWCGPCKMIAPILDEIADEYQGKLTVAKLNIDQNPGTAPKYGIRGIPTLLLFKNGEVAATKVGALSKGQLKEFLDANLAGSGSGVSGVDLGTENLYFQSASAVEDIRKVLSDSSSPVAGQKYDYILVGGGTAACVLANRLSADGSKRVLVLEAGPDNTSRDVKIPAAITRLFRSPLDWNLFSELQEQLAERQIYMARGRLLGGSSATNATLYHRGAAGDYDAWGVEGWSSEDVLSWFVQAETNADFGPGAYHGSGGPMRVENPRYTNKQLHTAFFKAAEEVGLTPNSDFNDWSHDHAGYGTFQVMQDKGTRADMYRQYLKPVLGRRNLQVLTGAAVTKVNIDQAAGKAQALGVEFSTDGPTGERLSAELAPGGEVIMCAGAVHTPFLLKHSGVGPSAELKEFGIPVVSNLAGVGQNLQDQPACLTAAPVKEKYDGIAISDHIYNEKGQIRKRAIASYLLGGRGGLTSTGCDRGAFVRTAGQALPDLQVRFVPGMALDPDGVSTYVRFAKFQSQGLKWPSGITMQLIACRPQSTGSVGLKSADPFAPPKLSPGYLTDKDGADLATLRKGIHWARDVARSSALSEYLDGELFPGSGVVSDDQIDEYIRRSIHSSNAITGTCKMGNAGDSSSVVDNQLRVHGVEGLRVVDASVVPKIPGGQTGAPVVMIAERAAALLTGKATIGASAAAPATVAA

SEQ ID NO: 4 - protein, 15 aa, artificial sequence
  Consensus sequence
  MISC_FEATURE (2)..(2): X is any amino acid
  MISC_FEATURE (4)..(7): X is any amino acid
  MISC_FEATURE (9)..(9): X is D or E
  MISC_FEATURE (10)..(10): X is any amino acid
  MISC_FEATURE (12)..(12): X is A or G
  MISC_FEATURE (14)..(14): X is any amino acid
  MISC_FEATURE (15)..(15): X is K or R
GXLXXXXCXXGXFXX

SEQ ID NO: 5 - protein, 580 aa, Chlamydomonas reinhardtii
LSVRAAAGPAGSEKFDYVLVGGGTASCVLANKLSADGNKKVLVLEAGPTGDAMEVAVPAGITRLFAHPVMDWGMSSLTQKQLVAREIYLARGRMLGGSSGSNATLYHRGSAADYDAWGLEGWSSKDVLDWFVKAECYADGPKPYHGTGGSMNTEQPRYENVLHDEFFKAAAATGLPANPDFNDWSHPQDGFGEFQVSQKKGQRADTYRTYLKPAMARGNLKVVIGARATKVNIEKGSSGARTTGVEYAMQQFGDRFTAELAPGGEVLMCSGAVHTPHLLMLSGVGPAATLKEHGIDVVSDLSGVGQNLQDHPAAVLAARAKPEFEKLSVTSEVYDDKCNIKLGAVAQYLFQRRGPLATTGCDHGAFVRTSSSLSQPDLQMRFVPGCALDPDGVKSYIVFGELKKQGRAWPGGITLQLLAIRAKSKGSIGLKAADPFINPAININYFSDPADLATLVNAVKMARKIAAQEPLKKYLQEETFPGERASSDKDLEEYIRRTVHSGNALVGTAAMGASPAAGAVVSSADLKVFGVEGLRVVDASVLPRIPGGQTGAATVMVAERAAALLRGQATIAPSRQPVAV

SEQ ID NO: 6 - protein, 611 aa, Chlamydomonas reinhardtii
MMLGPKTVTRGATKGAAPRSMAARRVGGARRLSVRAAAGPAGSEKFDYVLVGGGTASCVLANKLSADGNKKVLVLEAGPTGDAMEVAVPAGITRLFAHPVMDWGMSSLTQKQLVAREIYLARGRMLGGSSGSNATLYHRGSAADYDAWGLEGWSSKDVLDWFVKAECYADGPKPYHGTGGSMNTEQPRYENVLHDEFFKAAAATGLPANPDFNDWSHPQDGFGEFQVSQKKGQRADTYRTYLKPAMARGNLKVVIGARATKVNIEKGSSGARTTGVEYAMQQFGDRFTAELAPGGEVLMCSGAVHTPHLLMLSGVGPAATLKEHGIDVVSDLSGVGQNLQDHPAAVLAARAKPEFEKLSVTSEVYDDKCNIKLGAVAQYLFQRRGPLATTGCDHGAFVRTSSSLSQPDLQMRFVPGCALDPDGVKSYIVFGELKKQGRAWPGGITLQLLAIRAKSKGSIGLKAADPFINPAININYFSDPADLATLVNAVKMARKIAAQEPLKKYLQEETFPGERASSDKDLEEYIRRTVHSGNALVGTAAMGASPAAGAVVSSADLKVFGVEGLRVVDASVLPRIPGGQTGAATVMVAERAAALLRGQATIAPSRQPVAV

SEQ ID NO: 7 - protein, 568 aa, Phaeodactylum tricornutum
YDYIICGGGLAGCVLAERLSQDESKRVLVLEAGGSDYKSLFIRIPAGVLRLFRSKYDWQHETGGEKGCNGRNVFLQRGKILGGSSCTNVCLHHRGSAEDYNSWNIPGWTATDVLPFFKQSQKDETGRDATFHGADGEWVMDEVRYQNPLSKLFLEVGEAAGLGTNDDFNNWSHPQDGVGRFQVSEVNGERCSGATAFLSKAAKRSNVIVRTGTMVRRIDFDETKTAKGITYDLMGDDTCTTFQACLKEGGEVLVTGGAIASPQLLMCSGIGPGKHLRSLGIPVVHDNSAVGENLQDHPAAVVSFKTPQKGVSVTSKLRLFGKTNPIPVFQWLFFKSGLLTSTGCDHGAFVRTSDSLEQPDLQIRFLAARALGPDGMTTYTKFRTMKTVEDGYSFQSVACRAKSKGRIRLSSSNSHVKPMIDGGYLSNQDDLATLRAGIKLGRMLGNRPEWGEYLGQEVYPGPDVQTDEEIDEYIRNSLHTANALTGTCKMGTGRGAVVGPDLRVIGVNGVRVGDSSVFPCIPGGQTATPTVMIGDRAAVFVRQPVSQLNIEIFREKGGTHPGATTASA

SEQ ID NO: 8 - protein, 614 aa, Phaeodactylum tricornutum
MKKSLRSLLVWTLSVSSASATTMAGAKPLGNVPRAQEDERKVVAEPYDYIICGGGLAGCVLAERLSQDESKRVLVLEAGGSDYKSLFIRIPAGVLRLFRSKYDWQHETGGEKGCNGRNVFLQRGKILGGSSCTNVCLHHRGSAEDYNSWNIPGWTATDVLPFFKQSQKDETGRDATFHGADGEWVMDEVRYQNPLSKLFLEVGEAAGLGTNDDFNNWSHPQDGVGRFQVSEVNGERCSGATAFLSKAAKRSNVIVRTGTMVRRIDFDETKTAKGITYDLMGDDTCTTFQACLKEGGEVLVTGGAIASPQLLMCSGIGPGKHLRSLGIPVVHDNSAVGENLQDHPAAVVSFKTPQKGVSVTSKLRLFGKTNPIPVFQWLFFKSGLLTSTGCDHGAFVRTSDSLEQPDLQIRFLAARALGPDGMTTYTKFRTMKTVEDGYSFQSVACRAKSKGRIRLSSSNSHVKPMIDGGYLSNQDDLATLRAGIKLGRMLGNRPEWGEYLGQEVYPGPDVQTDEEIDEYIRNSLHTANALTGTCKMGTGRGAVVGPDLRVIGVNGVRVGDSSVFPCIPGGQTATPTVMIGDRAAVFVRQPVSQLNIEIFREKGGTHPGATTASA

SEQ ID NO: 9 - protein, 585 aa, Coccomyxa subellipsoidea
ALRVRAIIKSDNPAADKYDFILVGGGTAGCVLANRLTADGSKKVLLLEAGGANKAREVRTPAGLPRLFKSALDWNLYSSLQQAASDRSIYLARGKLLGGSSATNATLYHRGTAADYDAWGVPGWTSQDALRWFIQAENNCRGIEDGVHGTGGLMRVENPRYNNPLHEVFFQAAKQAGLPENDNFNNWGRSQAGYGEFQVTHSKGERADCFRMYLEPVMGRSNLTVLTGAKTLKIETEKSGGATVSRGVTFQVNGQDGSKHSAELAAGGEVVLCAGSIHSPQILQLSGIGPQAELRSKDIPVVADLPGVGQNMQDHPACLSAFYLKESAGPISVTDELLHTNGRIRARAILKYLLFKKGPLATTGCDHGAFVKTAGQSEPDLQIRFVPGLALDPDGIGSYTAFGKMKDQKWPSGITFQLLGVRPKSRGSVGLRSDDPWDAPKLDIGFLTDKEGADLATLRSGIKLSREIAAEPAFGAYVGNELHPGAAASSDSAIDSFIRDTVHSGNANVGTCSMGVNGNAVVDPSLRVFGIRGLRVADASVIPVIPGGQTGAATVMVAERAAEILLGSNQKQPAAAVPAAQPALA

SEQ ID NO: 10 - protein, 580 aa, Volvox carteri
PVAVKAAASVGSEKFDYILVGGGTAGCVLANKLSANGSKKVLVLEAGPTGDAMEVAVPAGIARLFAHPVFDWGMSSLTQQQLVAREIYLARGRLLGGSSGTNATLYHRGTPADYDSWGLEGWTSKDLLDWFVKAECYGDGPRAFHGQSGSMNVEQPRYQNVLHDEFFRAAAAAGLPANEDFNDWSRPQEGYGEFQVAQKNGERADTYRTYLKPAMGRDNLKVMTGARTTKVHIEKSSTGPRARGVEYATQQFGERYTAELTPGGEVLMCTGAVHTPHLLMLSGIGPAPTLLEHGLDVISSLPGVGANLQDHPAAVLAVRAKPEFEGLSVTSEIYDSKCNIRLGAVMKYLFGRRGPLATTGCDHGAFVRTSASHSQPDLQMRFVPGCALDPDGVKSYIVFGELKKQGRAWPGGITLQLLGIRAKSRGSIGLKAADPFINPAININYFSDPEDLATLKNGVRIAREIVAQEPLRKYLLEETFPGERANTDKDIEEYVRRTVHSGNALVGTCAMGTTPASGAVVSSADLKVFGVDGLRVVDASVLPRIPGGQTGAATVMVAERAAAMLLGQATITSRREPAAV

SEQ ID NO: 11 - protein, 557 aa, Ectocarpus siliculosus
VPAARYATSSVSMSVAEEGHKFIIIGGGTAGCVLANRLSADKDNSVLVLEAGSEKFNDRNIKMPIAILRLFKSVFDWGFQSENEKFATGDGIYLCRGKVLGGSSCTNVMLYHRGEEADYDAWGVDGWKGKDVLPYFKKAENNRSKKKGEFHGKGGLMQVENARYMNPLTKLFFKACEQAGLSENEDFNDWSHSQEGFGRFQVAQKRGKRCSAASSYLKEAMGRKNLDVQTSAQITKVLIENGGAIGVEYVRDGEKKIAKLAVGGEILLAGGAISSPQVLMLSGVGPAEHLRSKGIEVKSNVPGVGKNLRDHPAVTVMADINKPISITDKVLKEGSGDVNKITALQWLLTGTGPLTSPGCENGAFFKTTPDKAAADLQLRFVPGRSTTPDGVKAYNTIGTKGRPPSGVTVQVVGIRPQSEGHVELRSSDPFDKPHIVTNYLESGEDMASLTNGIEMARKLFDQEAFGEMVDKEVFPGRDNKEISEYIKSTVHSANALVGTCKMGEESDNMSVVNSALKVKGVAGLRVIDSSVMPSIPGGQTAAPTIMIAEKAADMLMA

SEQ ID NO: 12 - protein, 601 aa, Emiliania huxleyi
LRGGSGVTGGSLGRGGGSPAIDGEFDYIIVGGGAAGCVLANRLSADPAHRVLLIEAGGDASRDKRAQVPWAFTKLLRSEYDWDFHVEAEAAVNQQEVYLCRGKALGGSSVTNVMLYHRGSPADYDAWEEAGARGWGAKDVLPYYLRVEDYGDGASQYHAVGGHVSVQEVPYQNQLSATFLRAMGQLGFRPNGDFNDWSSPQEGYGRYKVTQRAGRRCTAADGYLAAARERANLVVVTGAQATRLALDSAYDGAGRLQVSGVEFARGDEREPCSVRLARGGEAVLCAGAVQTPHLLLLSGIGPAEHLREVGVPVRADLPGVGSGLQDHPAVVVSYESKKAVAATDDALLKGYASLVNPLAMLRWLLFGRGPLACAACDHGGFVRSSPDLDQPDVQIRFVPARASSASGMNTLIELGRRARFLPGFSTQVVACRPRSEGRVRLRSADPFAKPIIEGIHLGAAEDVASLRHGIRLGRQVCAAAAFDEYRGEEVFPGAAVQSDEQIDEYIRSSVHSANALTSSCRMGDPSDPAAVLDSHLRVRGVGGLRVADASAMPRIIGGQTQAPTYMLAERAADILLHARLQAHEPATESVSQRLEVAAAAL

SEQ ID NO: 13 - protein, 533 aa, Aureococcus anophagefferens
LSEDPSKKVLVLEAGDRGPNSPLVKIPVAILKLFKSAYDWNFATRPSEAVADRSLYVCRGKGLGGSSLTNVMLYNRGSANDYDAWAAACGDDSWGAEEMLGYFKKAEDCLVPAHRANHYHGVGGPYASSHVPYTNEMSTAFVEAAVEDGGVRNGDFNDWSTSQVGFGRFAVSQRKGARVDAATAYLPRKVRRRANLDVVRGAALSGVTWNANKATGVEFAFGGVSGIACGGEVILSGGAVHSPQMLMLSGVGAKAQLEEFGIPVVADRPGVGKNLQDHPACLVSWRGSAKAQGKSHSTQLRIPGTTKTSPKALLQWLFLGRGPLASPGCDHGGFAKVGAGDGDCDVQFRFLATKSITPDGMSTISDSYEAAVDHPDGLTIQTIVARPKSRAGEVKLASRDPAAKPVIENAYLSDEADVMTMVKALQKARSIASRAPLSAYAGHEEFPGEDVADERQLAAYVRNTAHTANAVVGTCKMGESSDALAVVDNHLKVIGVSNLRVVDASVMPTLPGGQTAASTVALAEKAADLIKGG

SEQ ID NO: 14 - protein, 1236 aa, Nannochloropsis gaditana
LSKTTIGLQSFVTANYGVRRAISLRGGLQSVSMKAPAAVASSTYDYIIVGGGIGGCVLANRLTESGRFKVLLLEAGKSAERNPYVNIPAGVVRLFKSALDWQFESAPERHLDGKEVYLVRGKAMGGSSAVNVMLVHRGSASDYAKWEAEGAQGWGPEEALRYFKKMEDNLVGGEGRWHGQGGMYPVDDVKYQNPLSKRFLQACEEYGWRANPDFNDWSHPQDGYGSFKVAQKHGKRVTAASGYLNKAVRRRPNLDILSEALVTRVLLEGEGDVKAVGVEFTGKDGKTHQVRTTGKAGEVLLAGGAVNSPQLLMLSGIGPEADLQAVGIATKVNRPGVGENLQDHPAVTIAHNITRPISLCDDLFLFHTPVPKPHQVLRWTLTGSGPLTTPGCDHGAFLKTREDLQEPNVQFRFIAGRGSDPDGVRSYIMGGSARPLSGLTLQVVNIRPKSKGKLTLASKDPLKKPRIEVRYLSAAEDLQALRTGMRIGRDLIKQRAFADILDEEVFPGPAAQTDEELDAYIRDSLHTANALVGTCKMGSVEDRNAVVDPECRVIGVGGLRVVDASVMPVIPGGQTGSGTTMLAEKAADLVRAHAGDLVEMGVQDEERKGGWFNGLLGRKQKVATEKERGERGKSERFVSEVIRHMGRVFVQVSRARRAQTCMRVGKGLDRERQLECAMRKELTIALFYAMLFTMRHSGFLSTTGRASYKDLGYLTGSCRAHPCTSPSSLCLFPEKPFMKLSPALAVVGFCFNSINVQGFLLSNLAGRSLKHPVPQKGLYSRIEYDAREPRLDEFGLPLDPADLMEKPRVPLKDRVYHIIDMTNDWVDAVSRGRREEETRRIIQRRRAAAKAMAIKDKVLISLDYVFHPVKAWRTFVADPLEARHQRQLRQQAEKRARLERYLQRYNTVKNRFHDTLDLLESTTRTSVKVAKSVSSAVVGAPGTVTRTVKEVKSQAQGTAEAVAKVSSSVSSVVSKITSVIRKEDGALAGAKGKKDPRSEDEGKADPVKVREIWETKEQTAIRTIWEADELVTPVTPPATAMASTVSVSEPQDENEASISQGAAPSPSTSSPSSPEPVTRLSFRARVEADEKERFGSRRLKISGNVPPTASPTRGASSLPLDTLSSSATQTFERSKVGPPIRTSKARCIGKCVHNGWKGICEEWFVHISFPTYAVSIVRPPMHVHNFKVICCVLAVRHARRKKEMSTALSTHLIYLLLKTVKMLQDLPQLRRKGKTN

SEQ ID NO: 15 - DNA, 1785 bp, Chlorella variabilis
cgcgcctctgcggtggaggacatccgcaaggtgctgtctgacagcagcagcccggtggcggggcagaagtacgactacattctggtcggcggcggcaccgcggcctgcgtgctggccaatcgcctgtccgccgacggctccaagcgtgtgctggtgctggaagccggccccgacaacacctcgcgcgacgtcaagatccccgccgccatcacccgcctcttccgcagccccctcgactggaacctcttctccgagctgcaggagcagctggcggagcgccagatctacatggcgcgcggccggctgctgggcggcagcagcgccaccaatgccacgctgtaccaccgcggcgcggcgggcgactatgatgcctggggcgtggagggctggagctcggaggacgtgctcagctggtttgtgcaggcggagaccaacgccgactttggccctggcgcgtaccacggcagcggcggccctatgcgtgtcgagaacccacgctacaccaacaagcagctgcacaccgccttcttcaaggccgcagaggaggtggggcttaccccaaacagcgatttcaacgactggagccacgatcatgctgggtacggtaccttccaggtcatgcaggacaagggcacacgtgccgacatgtaccggcagtacctcaagcccgtgctgggccgcagaaacctgcaggtgctgaccggcgcggccgtgaccaaggtcaacattgaccaggctgcaggcaaggcgcaggctctgggtgtggagttctcaaccgacgggcccacaggtgagcggctgagcgctgagctggcgccaggcggcgaggtgatcatgtgtgccggcgccgtgcacacgcccttcctgctcaagcacagcggcgtggggccctcggcggagctcaaggagtttggcatcccggtggtttccaacctggcaggtgtgggtcagaacctgcaggaccagcccgcctgcctgaccgcggcgccggtcaaggaaaagtatgatggcatcgccatcagcgaccacatctacaacgagaagggccagatccgcaagcgcgccattgccagctacctgctgggcggccgcggcggcctcacatccaccggatgcgaccgcggcgcctttgtgcgcacggcaggccaggcgctgccagatctgcaggtgcgctttgtgccgggcatggcgctggacccggatggcgtgtccacgtatgtgcgctttgccaagttccagtcccaggggctcaagtggcccagcggcatcaccatgcagctgatcgcctgccgcccgcaaagcacgggcagcgtgggcctcaagagtgccgacccctttgcgccgcccaagctgagccccggctatctgacggacaaggacggcgctgacctggccacgctccgcaagggcatccactgggcgcgcgacgtggcgcgcagcagcgcgctcagcgagtacctggatggcgagctgttccccggcagcggagtggtgagcgatgatcagattgatgagtacatccgccgcagcatccatagctccaacgccatcacaggcacatgcaagatgggcaatgccggcgacagcagcagcgtggtggacaaccagctgcgggtgcacggtgtggagggcctgcgggtggtggatgcctcggtggtgcccaagatcccaggtggccagacgggcgcgccagtggtgatgattgcggagcgcgccgccgcgctgttgactggcaaggcgacgatcggggcgagcgctgcggccccggcgacagtggcagcatga

SEQ ID NO: 16 - DNA, 1743 bp, Chlamydomonas reinhardtii
ctgtcggtgcgtgctgctgcgggcccagctggctcggagaagttcgactacgtgcttgtcgggggtggcactgcctcgtgcgtgcttgctaacaagctgtcggctgatggaaacaagaaggttctggttctggaggctggccctaccggtgacgccatggaggtggctgtgcccgccggcatcacccgcttgttcgcgcacccagtgatggactggggcatgtcgtcgctgacacagaagcagctggtggcccgcgagatctacctggcccgcggccgcatgctgggcggctcctccggctctaacgccacgctgtaccaccgcggcagcgccgccgactacgacgcttggggcctggagggctggagcagtaaggacgtgctggactggttcgtcaaggcggagtgctacgccgacggccccaagccctaccacggcactgggggcagcatgaacacggagcagccgcgctacgagaacgtgctgcacgatgagttcttcaaggccgccgccgccaccggcctgcccgccaaccccgatttcaacgactggagccacccgcaggacggcttcggtgagttccaggtgtctcagaagaagggccagcgcgccgacacctaccgcacctacctcaagcccgccatggcgcgcggcaacctcaaggtggtgattggtgcccgggccaccaaggtcaacattgagaagggctcgtcgggcgcacgcacgaccggcgtggagtacgccatgcagcagttcggcgaccgcttcaccgccgagctggcccctggcggcgaggtgctgatgtgctcgggcgcggtgcacacgccgcacctgctcatgctgtcgggcgtgggccccgccgccacgctgaaggagcacggcatcgatgtggtgtcggacctgtcgggtgtggggcagaacctgcaggaccaccccgcggcggtgctggcggcgcgcgccaagccagagtttgagaagctgtcggtgaccagcgaggtgtatgacgacaagtgcaacatcaagctgggcgccgtggcgcagtacctgttccagcgccgcggcccgctggccaccaccggctgcgaccacggagccttcgtgcgcacctcctcctcgctctcgcagcccgacctgcagatgcgcttcgtgccgggctgcgccctggaccccgatggcgtcaagtcctacatcgtgtttggcgagctcaagaagcagggccgcgcatggcccggcggcatcacgctgcagctgctggccatccgcgccaagagcaagggcagcatcggcctgaaggcggctgacccgttcatcaaccccgccatcaacatcaactacttctccgaccccgccgacctggccacgctggtcaacgccgtcaagatggcgcgcaagatcgcggcgcaggagccgctcaagaagtacctgcaggaggagacgttccccggcgagcgcgcctccagcgacaaggacctggaggagtacatccgccgcaccgtgcactcgggcaacgcgttggtgggcaccgcggccatgggcgcctcgcccgcggccggcgccgtggtgtcctccgccgacctcaaggtcttcggcgtggagggcctgcgtgtggtggacgcctcggtgctgccgcgcatccccggcggccagaccggcgccgccactgtcatggtggcggagcgcgcggcggcgctgctgcgcggccaggccaccatcgcgcccagccgccagcccgtggccgtgtaa

SEQ ID NO: 17 - DNA, 1707 bp, Phaeodactylum tricornutum
tacgactacattatctgcgggggagggttggctgggtgcgttttggctgaacgcctttcgcaggacgagtccaagcgtgtgctcgtactagaggctggcggctcggactacaaaagtcttttcatcaggattccggctggagtcttacggctctttcgcagtaaatacgattggcaacatgaaacgggcggtgaaaagggttgcaacggacggaatgtgtttttgcaacgcggcaagattctcggcggatcttcgtgcaccaatgtatgtctgcatcaccgtgggtcagcggaagattacaacagctggaacattcccgggtggacggctactgatgtgcttcctttcttcaagcaatcgcaaaaggatgagacgggccgggatgccacgttccacggtgcggatggggagtgggtcatggatgaggtgcgataccaaaatccattgagcaagttattcctggaggtaggggaggcagctggcctcggaaccaatgatgatttcaacaactggtcgcatccgcaggatggcgttgggcgcttccaggtttcagaagtaaacggagaacgatgttcgggagccacagcatttctaagtaaagcggccaagcgctcaaatgtcatagttcgaactggcactatggtgagaaggatcgactttgatgagacaaaaacagcgaaagggattacctacgatttgatgggcgatgacacatgtacgacatttcaagcttgtttgaaagagggtggcgaagtgctggtgacaggtggagcaattgcatcccctcagcttctcatgtgctccggaattggacctggcaagcacttacggtcgctgggcattccagtagtccacgacaactcggcagttggtgagaacctgcaggatcacccagctgctgtcgtttcctttaaaacccctcaaaagggagtttctgttacttctaaattgcggctcttcggtaagacaaaccccattccagtcttccagtggctattttttaaaagtggtcttttgacctccactggatgcgatcatggcgctttcgttcggacatcggattcactcgaacaaccggacttgcagattagattcttggcagctcgcgctcttggacccgacggaatgaccacgtataccaaattccgtacgatgaaaacagttgaagatggttattcgttccagagtgttgcatgtcgagcaaaaagcaagggaaggattcggttatcttcgtccaactcgcacgtaaagcctatgattgatggcggatacctctctaaccaggatgatcttgccacactacgtgctggtatcaagcttggacgtatgctcggtaaccgaccggaatggggcgagtaccttggtcaagaggtgtatccagggccagatgtgcaaacggatgaagagattgacgaatacattcgtaactcgctccataccgccaatgctttaacggggacatgcaaaatgggaacgggtcgtggggctgttgttgggcccgatttacgtgtaattggggtcaatggtgtacgtgtgggggattcatctgttttcccctgcattccagggggacaaacggcaacaccgaccgtcatgataggggatcgggccgctgtttttgttcggcaacccgtatcccagctgaacattgaaattttcagagaaaaagggggcacacatcctggggcaacgaccgcctcagcctag

SEQ ID NO: 18 - DNA, 1758 bp, Coccomyxa subellipsoidea
gcactgcgggtcagggcgataatcaaaagcgacaatccagctgcagataagtatgacttcatcctggtcggcggcggcacagcaggctgcgtgctggccaacaggctgacagcagatggatccaagaaggtcctgctgctcgaggcgggaggcgccaacaaggcgcgggaggtacgcacaccggccgggctgccgcgcctgttcaagagcgccctcgactggaacctctactcctccctgcagcaggcagccagcgacagatcgatctacctggcacggggaaagcttctgggtggcagctccgcaactaatgccacgctgtaccaccgggggactgcggcagactacgacgcgtggggtgtgccggggtggacctcccaggacgccctgcgctggtttattcaggcagagaacaactgcagagggattgaggacggggtgcatgggaccgggggattgatgcgcgtggagaaccctcgctacaacaaccccctgcacgaggtctttttccaggcggccaagcaggccggcctcccagagaacgacaactttaacaactggggcagatcacaggcggggtacggggagttccaggtgactcacagcaagggtgagcgcgccgactgcttccggatgtacctggagccagtcatggggcgttccaacctcacagtgctcaccggagccaaaacgctcaaaatcgaaactgaaaagtccggcggcgccacggtctcgcgcggcgtcaccttccaggtcaacggccaggacggcagcaagcactcagctgagctggcggctggcggcgaggtggtgctgtgcgcggggtcaatccactcgccccagatcctgcagctctccggcatcggcccccaggcggagctgcgctccaaggacatccctgtcgtcgcagacctgcccggcgtcggccagaatatgcaggaccacccggcgtgcctgtcagccttctacctcaaagagagcgcgggtcccatcagtgtgactgatgagttgctgcacaccaatggccgaatccgcgcgcgcgcaatcctaaagtacctgctcttcaaaaaggggcccctcgccaccacaggatgcgaccacggcgcctttgtgaagactgcaggtcagagtgagccggacctgcagatccgctttgtgccgggtctggcgcttgaccctgacggcatcggatcctacacggcctttggcaagatgaaggaccagaagtggccctccggaatcaccttccagctgctcggagtgcggcccaagagccgcgggtcggtgggtcttcgcagcgacgacccctgggacgcgccaaaactggacatcggcttcctgactgacaaggagggcgctgacctggccacgctgaggagcggcatcaagctctcgcgcgagatcgcagcggagccggcattcggagcatatgtaggcaacgaacttcacccgggcgcagccgcctcgtccgattctgcgatcgactcattcatccgtgacacggtgcactcgggcaatgccaacgtgggcacatgctcgatgggggtgaatgggaacgccgtcgtggacccgtcactcagagtgttcggcatccgcggcctgcgagtggccgacgcatcagtcatccccgtcatcccaggaggccagaccggcgctgcaacggtgatggtggcagagagggccgcggagattctcctcggctcgaaccagaagcagccggccgccgccgtccccgccgcgcagccggccctggcttga

SEQ ID NO: 19 - DNA, 1744 bp, Volvox carteri
tccagttgcagtcaaagctgcggcaagcgtggggtcggagaagttcgactacatccttgtgggaggagggacggcaggttgcgttctggcaaacaaattgtccgctaatggcagcaagaaggttcttgttcttgaggctggtccaaccggcgatgctatggaagtggccgtaccggccggtattgcccgtctctttgcacatccagtttttgactggggtatgtccagtttgacgcagcagcagctggttgcacgcgagatctaccttgctcgcggtcgccttctgggcggttcctctgggaccaacgcaacgctgtatcatcgcggcacccccgctgactacgacagttggggcttggagggctggacgagcaaggatctacttgattggttcgttaaggccgaatgctatggagacggtccccgggccttccatggccagtccggttctatgaatgtggagcaaccgcgttaccagaacgtcctgcacgacgagtttttcagggctgctgcggcagctggattacctgccaacgaggatttcaatgactggagccggccgcaggagggctatggggagttccaggtggcccagaagaacggtgagcgcgcggacacgtatcggacctacctcaagccggctatgggccgcgacaacctgaaggtgatgaccggcgcgcgtacgaccaaagtgcatatcgagaagagctcgacgggtccacgtgcccgcggtgtcgagtatgctacccagcaatttggggagcgctacaccgccgagctgactcctggtggcgaggttctcatgtgcaccggtgccgtgcacacaccgcacctactgatgctttcgggcattgggccggcgccgaccctccttgagcacggactcgacgtgatatcaagcctgcctggcgtgggtgccaacctgcaggatcacccagccgcggtgcttgctgtccgggctaagcccgagttcgagggactgtcggtcacttcggaaatctatgacagcaagtgcaacatccggttgggcgccgttatgaagtacctgttcggacgccgcgggccacttgcaaccacaggctgtgatcatggcgcttttgtgcgcacttcggcctcgcattcgcagccggacctgcagatgcgattcgtgcccggttgcgcgctggaccccgacggcgtgaagtcgtacattgtgttcggcgagctgaagaagcagggccgtgcttggcccggcggtatcacgttgcagctgctgggcatccgcgccaagagcaggggcagcatcggtctcaaggccgcggatcccttcatcaaccccgccattaacataaactatttctccgatcctgaggaccttgccacgcttaagaacggtgtgcgcattgcgcgcgaaatcgttgcccaggagccattgcgcaaataccttctggaggagaccttccccggggagcgggcgaacactgacaaggacattgaggagtatgtccggcgcacggtccacagcggcaacgcgcttgtgggcacctgcgcgatgggtaccacgccagccagtggcgccgtggtgtcttctgctgacctcaaggtgttcggtgttgacgggctgcgtgtcgtggatgcgtctgtgctgccacgcattccaggcgggcaaacaggagcggccactgtcatggttgcagagcgggcggcggccatgctgcttggacaggcgacgattacttctcgtcgcgagcctgcggctgtttag

SEQ ID NO: 20 - DNA, 1674 bp, Ectocarpus siliculosus
gtgcctgcagcacgttatgcgacgtcttcggtgagcatgtcggtggcggaagaaggccacaagttcatcatcatcggcgggggtacggctgggtgtgttctggcgaaccgcctctctgccgacaaggacaattcagtgctggtgttggaggccggctcggaaaaattcaatgacaggaatatcaagatgcccatcgcaatcctaaggttgttcaagtctgtcttcgactggggcttccagtcggaaaacgagaagtttgccaccggcgacggcatctacctctgccgtggcaaggtcctcggcgggtctagctgcaccaacgtcatgctttaccatcgcggagaggaggctgactatgacgcgtggggggtggatggatggaaaggcaaggacgtgctcccctacttcaagaaggcggagaacaaccgatccaagaaaaagggggagttccacggcaagggaggcctgatgcaggtggaaaacgcgcgttacatgaaccctttgacgaagttgttcttcaaggcgtgcgagcaggcaggcctgtcggagaacgaggacttcaacgattggtcccactcgcaggagggcttcggtcgcttccaggttgcacagaagagaggcaagcgctgttcggcagcctcctcctacctcaaggaagccatggggcgcaaaaacctggacgtgcagaccagcgcccagatcaccaaggtcttgatcgagaacggcggtgccataggcgttgagtacgtgcgggatggcgaaaagaagatcgccaagcttgccgtgggcggagagatcctgctagcaggaggtgccatcagctcaccgcaggtgctgatgctcagtggggtgggtccggccgagcacttgaggtccaagggcatcgaggtgaagagcaatgtgcctggggtcggaaagaacctccgcgaccatcccgctgtcaccgtgatggccgacatcaacaagcctatctccatcaccgacaaggttctcaaggagggctctggggacgtgaacaaaattacggcccttcagtggctgttgacgggaactgggccgctgacctcgccagggtgcgagaacggcgcgttcttcaagaccacgcctgacaaagcggcggcagatctgcagttgcgatttgtccctggaagatccactaccccagacggggtgaaggcgtacaacactattggcaccaaggggaggcctccttcgggtgtcaccgtgcaggtggtggggatccggccgcagagtgaaggccacgtcgagctgcgttcttcggacccgttcgacaagccacacatcgtcactaactaccttgagagtggggaggacatggcgtctttgacgaacggaatcgaaatggcacgaaagctgttcgaccaggaggccttcggagaaatggtggacaaagaagtcttccccggcagagacaacaaggagatctcggagtacatcaagtctaccgtgcactccgccaacgccttggttggcacttgcaagatgggcgaagaatcagacaacatgtctgttgtgaactcggcactcaaggtaaagggtgttgccgggctgagggtgatcgattcttcggtgatgccttcaatccccggcggtcaaacagcggcaccgacgatcatgatcgcagagaaagcggcggacatgctcatggcttag

SEQ ID NO: 21 - DNA, 1808 bp, Emiliania huxleyi
gccttcgcggcggcagcggcgtcactggcggcagcctcggccgcggcggcggctcgccggcgatcgacggcgagtttgactacatcatcgttggaggcggcgccgcgggctgcgtgctcgccaatcggctgagcgccgacccggcgcaccgggtgctgctgatcgaggccggaggcgacgcgtcgcgcgacaagcgtgcgcaggtgccgtgggccttcaccaagctgctgcgttccgagtacgactgggactttcacgtggaggcggaggcggcggtgaaccagcaggaggtgtacctctgccgcggcaaggcgctgggcggctcttcggtcacaaacgtgatgctctaccaccggggcagccccgcggactacgacgcttgggaggaggctggcgcgcgagggtggggcgcgaaggacgtgctcccgtattacctccgcgtcgaggactacggcgacggcgcctcgcagtaccacgccgtcggcgggcacgtctcggtgcaggaggtgccgtaccagaaccaactctcggcaaccttcctgcgggcgatggggcagctgggcttccggccgaacggagacttcaacgactggtccagcccgcaggaggggtacggccgctacaaggtgacccagcgggccggccgccgctgcaccgctgccgacggctacctggcggcggcgagagagcgcgcgaacctggtggtggtgaccggcgcgcaggcgacccgcctcgccctcgacagtgcgtacgacggcgcgggccggctgcaggtctccggcgtcgagtttgcacgcggcgacgagcgcgagccgtgctccgtccggctcgcgcgcggcggagaggccgtcctctgcgccggcgcggtccagacgccgcacttgctgctcctctccgggatcggcccggcggagcacctgcgcgaggttggcgtgccggtgcgggcggacctgcctggggtggggtccggcctgcaggaccaccccgcggtggtcgtctcgtacgagagcaagaaagcggtcgccgcgacggacgacgcgctcctcaagggctacgcgtcgctggtcaacccgctcgcgatgctgcgctggctcctgtttgggcgcgggccgctggcgtgcgccgcgtgcgaccacggcggcttcgtccgctcctcgcccgacctcgaccagcccgacgtccagatccgcttcgtgcctgcgcgcgcctcgtccgcctccgggatgaacacgctgatcgagctgggcaggagagcgcgcttcctgccgggcttctcgacgcaggtcgtcgcttgccgcccgcggagcgaggggcgcgtgcggctgcggtcggccgacccgttcgccaagccgatcatcgagggcatccacttgggcgcagcggaggacgtcgcgtcgctgcgccacggcatccggctcggccggcaggtttgcgccgcggcagccttcgacgagtaccgcggagaggaggtcttccccggcgcggcggtgcagtccgacgagcagatcgacgagtacatccgctcgtcggtgcactctgcgaacgcgctcacctcgtcctgccgcatgggcgacccgtccgacccggccgcagtcctcgactcccacttgcgcgtgcgcggcgtcggcggcttgcgcgtggccgacgcctccgccatgcctcgcatcatcggagggcagacgcaggcgcccacgtacatgctcgccgaacgtgccgccgacatcctgctgcacgcgcgcctgcaggcgcacgagccagccaccgagagcgtctcgcagcggctcgaggttgcggcggccgcactctag

SEQ ID NO: 22 - DNA, 1605 bp, Aureococcus anophagefferens
cgcctcagcgaggacccgagcaagaaggtgctcgtgctcgaggccggcgaccggggcccgaactcgccgctcgtgaagatccccgtggccatcctcaagctcttcaagtccgcgtacgattggaacttcgcgacgaggccgtccgaggccgtcgcggaccggagcctctacgtctgccggggcaagggcctgggcggcagctccctgacgaacgtcatgctctacaaccggggctcggccaacgactacgacgcgtgggcggccgcgtgcggcgacgactcgtggggggcggaagagatgctcggctacttcaagaaggccgaggactgcctcgtgccggcgcaccgagcgaaccactaccacggcgtcggcgggccctacgcgtcgagccacgtgccctacacgaacgagatgtcgacggcgttcgtcgaggccgccgtcgaggacggcggcgtgcgcaacggcgacttcaacgactggtccacgtcccaggtcggcttcggccgcttcgccgtgagccagcgcaagggggcaagggtggacgcggcgacggcctacctcccgcggaaggtccggcggcgcgcgaacttggacgtggtccgcggcgcggcgctctccggcgtcacgtggaacgcgaacaaggccacgggcgtcgagttcgccttcggcggcgtctcgggcatcgcctgcggcggcgaggtgatcctctccggcggcgcggtccactcgccgcagatgctcatgctctccggcgtcggcgcgaaagcgcagctcgaggagttcggcatccccgtcgtcgcggaccggccgggcgtgggcaagaatttgcaggaccacccggcctgcctcgtgtcctggcgcgggtcggccaaggcccagggcaagagccactcgacgcagctccggatccccgggacgacgaagacctcgcccaaggcgctcctccagtggctcttcctcggccggggccccttggcctcgccgggctgcgaccacggcggcttcgccaaggtcggcgccggcgacggcgactgcgacgtccagttccggttcctcgcgacgaagtcgatcacgcccgacggcatgtctaccatctccgactcctacgaggccgccgtggaccaccccgacggcttgacgatccagaccatcgtcgcccggcccaagagccgcgcgggcgaggtgaaactcgcgtcccgggacccggcggcgaagcccgtcatcgagaacgcgtacctctccgacgaggccgacgtcatgaccatggtcaaggcgctccagaaggcgcggtccatcgcgagccgggcgccgttgagcgcctacgcgggacacgaggagttcccgggggaggacgtcgcggacgagcgccaactggcggcctacgtgcggaacaccgctcataccgcgaacgcggtcgtcgggacctgcaagatgggcgagtccagcgacgccctcgccgtcgtcgacaaccacctcaaggtcatcggcgtctcgaacctgcgggtggtggacgcgtcggtgatgccgacgctgccgggcggccagacggccgcgtcgaccgtcgcgctcgcggagaaggccgcggacctcatcaaggggggctga

SEQ ID NO: 23 - DNA, 3711 bp, Nannochloropsis gaditana
ctctccaagaccaccatcggcctccaatccttcgtgacagcaaattatggagtgaggagagcaatctctctccgaggggggctacaatctgtttcgatgaaggcaccggctgccgttgcttcgtccacctacgactacatcatagtcggtggcggcatcggcggttgtgttctcgccaaccgactgacagaaagcgggcgtttcaaggtccttctcctggaggccggaaaatcagcagagcgaaacccgtacgtgaacatccccgcgggcgtggtccgcctctttaaatcggccttggattggcagtttgagagcgcccccgaaagacacctggacgggaaggaggtgtacttggtcagggggaaggccatgggaggctccagtgcggtgaatgtgatgctcgtacaccgcggctcggcctccgactacgcgaagtgggaggcggagggagctcagggatggggcccggaggaagccttacgctacttcaagaaaatggaagacaacttggtgggcggggaagggcggtggcacggccaggggggcatgtacccggtggacgacgtcaagtaccaaaaccctttgtccaagcgctttttacaggcgtgcgaggagtacgggtggcgggcgaacccggattttaacgactggtcccatccccaggacggatacgggagcttcaaagtggcgcagaagcacggcaaacgggtgacggccgcctccgggtacttgaacaaggccgttcgacgtcgaccaaacctagacattctgtcagaggcccttgtgacccgggttttgcttgagggagagggggatgtgaaggcggtcggggtggagttcacgggcaaagatgggaagacgcaccaggttcggaccacggggaaggcgggagaagttctcttggcgggcggcgcggtcaacagcccccaactcctgatgctgagtgggatcggacccgaggcagacctccaggcagtaggcatcgcgaccaaagtaaaccgtccgggcgtgggggagaacttgcaagaccatcccgccgtcactattgcgcacaacatcacgcgccctatctcgctctgcgacgacctcttccttttccacacacctgtccctaagccccaccaggtgctccggtggaccttgaccggatcgggcccgctgaccaccccaggctgcgaccacggcgcgttcctgaagacccgagaagacctccaggaacccaacgtacagtttcgtttcatagccgggcggggttcggaccctgacggcgtgcgctcctacatcatgggaggctcagcacgccccctgtcgggattgacgcttcaagtcgtcaacatccgccccaaaagcaaagggaagctgaccttggcgagcaaggacccgttgaagaagccccggatcgaagtccggtacttgtccgcggccgaagacttgcaggcccttcgcacgggcatgaggattggccgggatctgatcaagcaacgggcttttgcggatatcttggacgaggaagtgttcccggggcccgccgctcagacggacgaggaactggacgcctacatccgggatagcttgcacacggccaacgccctggtaggcacctgcaagatggggagtgtggaggatcggaacgcagtggtggacccggagtgccgggtcatcggcgtgggaggcctgcgggtggtggatgcaagcgtgatgcccgttatccccggagggcaaacgggaagtggcacgaccatgctggccgaaaaagcggccgacctggtcagggcccacgctggggatttggtggagatgggagtgcaagatgaggagaggaagggaggatggtttaacggcctgttagggcgcaaacagaaggtggcgacagaaaaggagcgaggcgaacgtggtaaaagcgaacgatttgtttctgaggtgattaggcatatgggtcgggttttcgtacaagtttcgagggcaaggcgtgcgcaaacgtgcatgagggtagggaagggtctcgatagggaacggcagttggagtgtgccatgcgcaaggaattgacgattgcgcttttttacgcaatgctttttacaatgagacatagtggatttctttcgacgactggtcgcgcctcatataaggaccttggatacttgacagggtcctgtcgcgcccacccttgtacatctccatcctccttgtgcctgtttccagaaaaacctttcatgaagctaagccctgctttggcggtcgttggcttttgctttaattctatcaatgtccaaggtttcctactcagcaaccttgccggtcggagcctgaagcatccggtcccacaaaagggcttgtatagtcgcattgagtacgatgcacgggagccacgtctcgatgaattcggcctccctcttgatccggcggatttgatggaaaaaccccgagtgcccctgaaggaccgagtttatcacatcattgacatgacaaacgactgggtcgatgctgtgagccgcggacggcgagaggaggagacgcgtcgcatcatccaacgacgtcgtgccgctgccaaggccatggcaatcaaggacaaggtcttgatttctcttgactacgtcttccatccagtcaaggcctggaggaccttcgtggcggaccccttggaagcacggcatcagcgccagctgcgtcagcaggcagaaaagcgagcgagactagaacggtatctgcaacgctataacacggtcaagaatcgcttccatgatactctggatcttttggagtcgacgacccggacatcggtgaaagtggccaagtccgtgagttccgcagtggtgggggcgcctgggacggtgacgcggaccgtgaaggaggtgaaaagccaggcacagggcacagcggaggcagtggcgaaggtgtcttcctccgtctcctcggtggtgtccaagatcacgtcggtgatcaggaaggaagacggggctctggcgggggccaaggggaaaaaggacccgagatcagaagacgaaggaaaagccgatccagtcaaggtccgggagatctgggaaacgaaagagcagaccgcgattcgcaccatctgggaagcggatgagcttgtcacgccggtaacaccgccagccacggctatggcgtcgacggtttcggtgtcagagcctcaggacgagaacgaagcttccatctctcagggagcggcgccttcccccagcacctcatcaccatcctcccccgagcccgtcacacgcctctctttccgggcacgtgtggaggcggacgagaaggaacgctttgggtcccgaagattgaagatatcggggaatgtcccgccgaccgcttctcccactcggggggcttcttctctccctttggacacgctttcctcctccgccacccaaacctttgagcgttccaaagtggggccgcccatacgaacaagtaaggcgagatgcattggaaaatgtgtacataacgggtggaaagggatatgtgaggaatggtttgtgcacattagttttccaacgtatgcggtctctatcgtccgtccacccatgcacgtgcataattttaaagtgatttgttgtgttctagcggtccgacatgcaagaaggaagaaggagatgagcacggctttatctacacatttaatttatttactgctgaaaacggtaaaaatgttgcaagatcttccccagctacggagaaagggcaaaacaaactag

SEQ ID NO: 24 - DNA, 20 bp, Artificial sequence
  primer
atggcgtcaattacatcgcg

SEQ ID NO: 25 - DNA, 18 bp, artificial sequence
  Primer
tcatgctgccactgtcgc

SEQ ID NO: 26 - protein, 15 aa, artificial sequence
  consensus sequence
  MISC_FEATURE (2)..(2): X is any amino acid
  MISC_FEATURE (4)..(7): X is any amino acid
  MISC_FEATURE (9)..(9): X is D or E
  MISC_FEATURE (10)..(10): X is any amino acid
  MISC_FEATURE (12)..(12): X is A or G
  MISC_FEATURE (14)..(14): X is any amino acid
  MISC_FEATURE (15)..(15): X is K, R, S or E
GXLXXXXCXXGXFXX

SEQ ID NO: 27 - DNA, 37 bp, artificial sequence
  primer
ctgtacttccaatcagccagcgcagttgaagatattc

SEQ ID NO: 28 - DNA, 41 bp, artificial sequence
  primer
tatccacctttactgttatcatgctgcaacggttgccggtg

SEQ ID NO: 29 - DNA, 33 bp, artificial sequence
  primer
tacttccaatcaatgatgctgggtccgaaaacc

SEQ ID NO: 30 - DNA, 41 bp, artificial sequence
  primer
tatccacctttactgttctactaaactgcaaccggctgacg

SEQ ID NO: 31 - DNA, 33 bp, artificial sequence
  primer
tacttccaatcaatgaaaaaaagcctgcgtagc

SEQ ID NO: 32 - DNA, 36 bp, artificial sequence
  primer
tatccacctttactgttctactatgcgcttgcggtg